European Patent Application EP 4 567 046 A1, published June 11, 2025. Title: ANTIBODY TARGETING EGFRVIII AND USE THEREOF IN CELL IMMUNOTHERAPY. Applicant: BEIJING DCTY BIOTECH CO., LTD. The sequence listing filed with the application follows.

SEQUENCE LISTING (198 sequences)

SEQ ID NO: 1 - protein, 5 aa, synthetic construct
DFSMH

SEQ ID NO: 2 - protein, 17 aa, synthetic construct
WINTETGEPSYADDFKG

SEQ ID NO: 3 - protein, 9 aa, synthetic construct
YGYDVRGDY

SEQ ID NO: 4 - protein, 5 aa, synthetic construct
DYYMH

SEQ ID NO: 5 - protein, 17 aa, synthetic construct
WIDPENGNTIYDPKFQG

SEQ ID NO: 6 - protein, 5 aa, synthetic construct
GWFAY

SEQ ID NO: 7 - protein, 5 aa, synthetic construct
DYSIH

SEQ ID NO: 8 - protein, 17 aa, synthetic construct
WINTETGEPTYADDFKG

SEQ ID NO: 9 - protein, 9 aa, synthetic construct
YGYDVRGDY

SEQ ID NO: 10 - protein, 5 aa, synthetic construct
DYYLH

SEQ ID NO: 11 - protein, 17 aa, synthetic construct
WIDPENGNTIYDPKFQG

SEQ ID NO: 12 - protein, 5 aa, synthetic construct
GYLTY

SEQ ID NO: 13 - protein, 5 aa, synthetic construct
RYWMH

SEQ ID NO: 14 - protein, 17 aa, synthetic construct
EINPSNGRANYNEKFMS

SEQ ID NO: 15 - protein, 10 aa, synthetic construct
GREITTGFAY

SEQ ID NO: 16 - protein, 5 aa, synthetic construct
DYYMH

SEQ ID NO: 17 - protein, 17 aa, synthetic construct
WIDPENGNTIYDPKFQG

SEQ ID NO: 18 - protein, 5 aa, synthetic construct
GYLVY

SEQ ID NO: 19 - protein, 5 aa, synthetic construct
DYYMH

SEQ ID NO: 20 - protein, 17 aa, synthetic construct
WIDPENGNTIYDPKFQG

SEQ ID NO: 21 - protein, 5 aa, synthetic construct
GYLAY

SEQ ID NO: 22 - protein, 5 aa, synthetic construct
DYYMH

SEQ ID NO: 23 - protein, 17 aa, synthetic construct
WIDPENGNTIYDPKFQG

SEQ ID NO: 24 - protein, 5 aa, synthetic construct
GWFAY

SEQ ID NO: 25 - protein, 5 aa, synthetic construct
DYYMH

SEQ ID NO: 26 - protein, 17 aa, synthetic construct
WIDPENGNTIYDPKFQG

SEQ ID NO: 27 - protein, 5 aa, synthetic construct
GYLVY

SEQ ID NO: 28 - protein, 5 aa, synthetic construct
DYYMH

SEQ ID NO: 29 - protein, 17 aa, synthetic construct
WIDPENGNTIYDPKFQG

SEQ ID NO: 30 - protein, 5 aa, synthetic construct
GWFAY

SEQ ID NO: 31 - protein, 5 aa, synthetic construct
DYYMH

SEQ ID NO: 32 - protein, 17 aa, synthetic construct
WIDPENGNTIYDPKFQG

SEQ ID NO: 33 - protein, 5 aa, synthetic construct
GYLVY

SEQ ID NO: 34 - protein, 5 aa, synthetic construct
DYYMH

SEQ ID NO: 35 - protein, 17 aa, synthetic construct
WIDPENGNTIYDPKFQG

SEQ ID NO: 36 - protein, 5 aa, synthetic construct
GYLVY

SEQ ID NO: 37 - protein, 5 aa, synthetic construct
NYAMS

SEQ ID NO: 38 - protein, 17 aa, synthetic construct
TITSGGSYTYYPDSVKG

SEQ ID NO: 39 - protein, 10 aa, synthetic construct
KDYGNYWFAY

SEQ ID NO: 40 - protein, 5 aa, synthetic construct
GYAMS

SEQ ID NO: 41 - protein, 17 aa, synthetic construct
TITSGGSYTYYPDSVKG

SEQ ID NO: 42 - protein, 10 aa, synthetic construct
KDYGNYWFAY

SEQ ID NO: 43 - protein, 5 aa, synthetic construct
GYAMS

SEQ ID NO: 44 - protein, 17 aa, synthetic construct
TITSGGSYTYYPDSVKG

SEQ ID NO: 45 - protein, 10 aa, synthetic construct
KDYGNYWFAY

SEQ ID NO: 46 - protein, 6 aa, synthetic construct
SGYSWH

SEQ ID NO: 47 - protein, 16 aa, synthetic construct
YIHYSGSTNYNPPLKS

SEQ ID NO: 48 - protein, 10 aa, synthetic construct
GVVSNYAMGN

SEQ ID NO: 49 - protein, 5 aa, synthetic construct
TYWMH

SEQ ID NO: 50 - protein, 17 aa, synthetic construct
YINPNTAYTEYNQNFKD

SEQ ID NO: 51 - protein, 12 aa, synthetic construct
GAYYRTYYAMDY

SEQ ID NO: 52 - protein, 5 aa, synthetic construct
NYGMN

SEQ ID NO: 53 - protein, 17 aa, synthetic construct
WINTYTGEPTYADDFKG

SEQ ID NO: 54 - protein, 11 aa, synthetic construct
EEFYSRGAMDY

SEQ ID NO: 55 - protein, 5 aa, synthetic construct
DYYIN

SEQ ID NO: 56 - protein, 17 aa, synthetic construct
WIYPGSGNTKYNEKFKG

SEQ ID NO: 57 - protein, 6 aa, synthetic construct
SSRCDF

SEQ ID NO: 58 - protein, 12 aa, synthetic construct
SASSSISSNYLH

SEQ ID NO: 59 - protein, 7 aa, synthetic construct
GTSNLAS

SEQ ID NO: 60 - protein, 9 aa, synthetic construct
HQGSSIPLT

SEQ ID NO: 61 - protein, 17 aa, synthetic construct
KSSQSLLNSSNQKNHLA

SEQ ID NO: 62 - protein, 7 aa, synthetic construct
FASTRAS

SEQ ID NO: 63 - protein, 9 aa, synthetic construct
QQHYSTPLT

SEQ ID NO: 64 - protein, 12 aa, synthetic construct
SASSGISSNYLH

SEQ ID NO: 65 - protein, 7 aa, synthetic construct
STSNLAS

SEQ ID NO: 66 - protein, 9 aa, synthetic construct
HQGSDIPLT

SEQ ID NO: 67 - protein, 17 aa, synthetic construct
KSSQNLLNSSNQKNYLA

SEQ ID NO: 68 - protein, 7 aa, synthetic construct
FASTRYS

SEQ ID NO: 69 - protein, 9 aa, synthetic construct
QQHYSTPLT

SEQ ID NO: 70 - protein, 11 aa, synthetic construct
KASQSVSNDVV

SEQ ID NO: 71 - protein, 7 aa, synthetic construct
YASNRYT

SEQ ID NO: 72 - protein, 9 aa, synthetic construct
QQDYSSPWT

SEQ ID NO: 73 - protein, 17 aa, synthetic construct
KSSQSLLNSSNQKNYLA

SEQ ID NO: 74 - protein, 7 aa, synthetic construct
FASTRES

SEQ ID NO: 75 - protein, 9 aa, synthetic construct
QQHYSIPLT

SEQ ID NO: 76 - protein, 17 aa, synthetic construct
KSSQSLLNSSNQKNYLA

SEQ ID NO: 77 - protein, 7 aa, synthetic construct
FASTRKS

SEQ ID NO: 78 - protein, 9 aa, synthetic construct
QQHYSTPLT

SEQ ID NO: 79 - protein, 17 aa, synthetic construct
KSSQSLLNSSNQKNHLA

SEQ ID NO: 80 - protein, 7 aa, synthetic construct
FASTRQS

SEQ ID NO: 81 - protein, 9 aa, synthetic construct
QQHYSTPLT

SEQ ID NO: 82 - protein, 17 aa, synthetic construct
KSSQSLLNSSNQKNYLA

SEQ ID NO: 83 - protein, 7 aa, synthetic construct
FASTRQS

SEQ ID NO: 84 - protein, 9 aa, synthetic construct
QQHYSTPLT

SEQ ID NO: 85 - protein, 17 aa, synthetic construct
KSSQSLLNSSNQKNHLA

SEQ ID NO: 86 - protein, 7 aa, synthetic construct
FASTRGS

SEQ ID NO: 87 - protein, 9 aa, synthetic construct
QQHYSTPLT

SEQ ID NO: 88 - protein, 17 aa, synthetic construct
KSSQSLLNSSNQKNYLA

SEQ ID NO: 89 - protein, 7 aa, synthetic construct
FASTRDS

SEQ ID NO: 90 - protein, 9 aa, synthetic construct
QQHYSTPLT

SEQ ID NO: 91 - protein, 17 aa, synthetic construct
KSSQSLLNSSNQKNYLA

SEQ ID NO: 92 - protein, 7 aa, synthetic construct
FASTRES

SEQ ID NO: 93 - protein, 9 aa, synthetic construct
QQHYSTPLT

SEQ ID NO: 94 - protein, 16 aa, synthetic construct
RSSQSLVHSDGNTYLH

SEQ ID NO: 95 - protein, 7 aa, synthetic construct
KVSNRFS

SEQ ID NO: 96 - protein, 9 aa, synthetic construct
SQSIHVPWT

SEQ ID NO: 97 - protein, 10 aa, synthetic construct
SASSSVSYMH

SEQ ID NO: 98 - protein, 7 aa, synthetic construct
STSNLAS

SEQ ID NO: 99 - protein, 9 aa, synthetic construct
QQRSSYPLT

SEQ ID NO: 100 - protein, 16 aa, synthetic construct
RSSQSLVHSDGNTYLH

SEQ ID NO: 101 - protein, 7 aa, synthetic construct
KVSNRFS

SEQ ID NO: 102 - protein, 9 aa, synthetic construct
SQTTQVPWT

SEQ ID NO: 103 - protein, 11 aa, synthetic construct
ITNTDIDDDMN

SEQ ID NO: 104 - protein, 7 aa, synthetic construct
EGNTLRP

SEQ ID NO: 105 - protein, 9 aa, synthetic construct
LQSDDLPLT

SEQ ID NO: 106 - protein, 15 aa, synthetic construct
KASQSVDYDGDSYMN

SEQ ID NO: 107 - protein, 7 aa, synthetic construct
AASNLES

SEQ ID NO: 108 - protein, 9 aa, synthetic construct
LQSNEDPYT

SEQ ID NO: 109 - protein, 16 aa, synthetic construct
RSSQFIVHSNGNTYLE

SEQ ID NO: 110 - protein, 7 aa, synthetic construct
KISNRFS

SEQ ID NO: 111 - protein, 9 aa, synthetic construct
FQGSHVPFT

SEQ ID NO: 112 - protein, 11 aa, synthetic construct
KASEDIYNRLA

SEQ ID NO: 113 - protein, 7 aa, synthetic construct
GATSLET

SEQ ID NO: 114 - protein, 9 aa, synthetic construct
QQYWSSPLT

SEQ ID NO: 115 - protein, 118 aa, synthetic construct
QIQLVQSGPELKKPGETVKISCKASGYTFTDFSMHWVKQAPGKGLKWMGWINTETGEPSYADDFKGRFAFSLETSASTAYLQINNLKNEDTATYFCANYGYDVRGDYWGQGTTLTVSS

SEQ ID NO: 116 - protein, 108 aa, synthetic construct
EIVLTQSPTTMAASPGEKITITCSASSSISSNYLHWYQQKPGFSPKLLIYGTSNLASGVPARFSGSGSGTSYSLTIGTMEAEDVATYYCHQGSSIPLTFGAGTKLELK

SEQ ID NO: 117 - protein, 114 aa, synthetic construct
EVQLQQSGAELVRPGALVKLSCKASGFNIKDYYMHWVKQRPEQGLEWIGWIDPENGNTIYDPKFQGKASITADTSSNTAYLQLSSLTSEDTAVYYCARGWFAYWGQGTLVTVSA

SEQ ID NO: 118 - protein, 113 aa, synthetic construct
DILMTQSPSSLAMSVGQKVTMSCKSSQSLLNSSNQKNHLAWYQQKPGQSPKLLVYFASTRASGVPDRFIGSGSGTDFTLTISSVQAEDLADYFCQQHYSTPLTFGAGTKLELK

SEQ ID NO: 119 - protein, 118 aa, synthetic construct
QIQLVQSGPELKKPGETVKISCKASGYTFTDYSIHWVKQAPGKGLKWMGWINTETGEPTYADDFKGRFAFSLETSASTAYLQINNLKNEDTATYFCSNYGYDVRGDYWGQGTTLTVSS

SEQ ID NO: 120 - protein, 108 aa, synthetic construct
EIVLTQSPTTMAASPGENITITCSASSGISSNYLHWYQQKPGFSPELLIYSTSNLASGVPARFSGSGSGTSYSLTIGTMEAEDVATYYCHQGSDIPLTFGAGTRLELK

SEQ ID NO: 121 - protein, 114 aa, synthetic construct
EVQLQQSGADLVRPGALVKLSCKASGFNIKDYYLHWVKQRPEQGLEWIGWIDPENGNTIYDPKFQGKASITADTSSNTAYLQLSSLTSEDTAVYYCARGYLTYWGQGTLVTVSA

SEQ ID NO: 122 - protein, 113 aa, synthetic construct
DIVMTQSPSSLAMSVGQKVTMNCKSSQNLLNSSNQKNYLAWFQQKPGQSPKLLVYFASTRYSGVPDRFMGSGSGTDFTLTVSSVQAEDLADYFCQQHYSTPLTFGAGTKLELK

SEQ ID NO: 123 - protein, 119 aa, synthetic construct
QVQLQQPGAELVKPGASVKLSCKASGYSFTRYWMHWVKQRPGQGLEWIGEINPSNGRANYNEKFMSKATLTVDKSSSTAYMQLSSLTSEDSAVYYCARGREITTGFAYWGQGTLVTVSA

SEQ ID NO: 124 - protein, 107 aa, synthetic construct
SIVMTQTPKFLLVSAGDRVTITCKASQSVSNDVVWYQQKPGQSPKLLIYYASNRYTGVPDRFTGSGYGTDFTFTITTVQAEDLAVYFCQQDYSSPWTFGGGTKLEIK

SEQ ID NO: 125 - protein, 114 aa, synthetic construct
EVQLQQSGAELVRPGALVKLSCKASGFNIKDYYMHWVKQRPEQGLEWIGWIDPENGNTIYDPKFQGKATITADTSSNTAYLQLSSLTSEDTAVYYCARGYLVYWGQGTLVTVSA

SEQ ID NO: 126 - protein, 113 aa, synthetic construct
DIVMTQSPSSLAMSVGQKVTMSCKSSQSLLNSSNQKNYLAWYQQKPGQSPKLLVYFASTRESGVPDRFIGSGSGTDFTLTISSVQAEDLADYFCQQHYSIPLTFGAGTKLELK

SEQ ID NO: 127 - protein, 114 aa, synthetic construct
EVQLQQSGAELVRPGALVKLSCKASGFNIKDYYMHWVKQRPEQGLEWIGWIDPENGNTIYDPKFQGKASITADTSSNTAYLQLSSLTSEDTAVYYCARGYLAYWGQGTLVTVSA

SEQ ID NO: 128 - protein, 113 aa, synthetic construct
DIVMTQSPSSLAMSVGQKVTMSCKSSQSLLNSSNQKNYLAWYQQKPGQSPKLLVYFASTRKSGVPDRFIGSGSGTDFTLTISSVQAEDLADYFCQQHYSTPLTFGAGTKLELK

SEQ ID NO: 129 - protein, 114 aa, synthetic construct
EVQLQQSGAELVRPGALVKLSCKASGFNIKDYYMHWVKQRPEQGLEWIGWIDPENGNTIYDPKFQGKASITADTSSNTACLQLSSLTSEDTAVYYCARGWFAYWGQGTLVTVSA

SEQ ID NO: 130 - protein, 113 aa, synthetic construct
DILMTQSPSSLAMSVGQKVTMSCKSSQSLLNSSNQKNHLAWYQQKPGQSPKLLVYFASTRQSGVPDRFIGSGSGTDFTLTISSVQAEDLADYFCQQHYSTPLTFGAGTKLELK

SEQ ID NO: 131 - protein, 114 aa, synthetic construct
EVQLQQSGAELVRPGALVKLSCKASGFNIKDYYMHWVKQRPEQGLEWIGWIDPENGNTIYDPKFQGKASITADTSSNTAYLQLSSLTSEDTAVYYCARGYLVYWGQGTLVTVSA

SEQ ID NO: 132 - protein, 113 aa, synthetic construct
DIVMTQSPSSLAMSVGQKVTMSCKSSQSLLNSSNQKNYLAWYQQKPGQSPKLLVYFASTRQSGVPDRFIGSGSGTDFTLTISSVQAEDLADYFCQQHYSTPLTFGAGTKLELK

SEQ ID NO: 133 - protein, 114 aa, synthetic construct; identical to SEQ ID NO: 117

SEQ ID NO: 134 - protein, 113 aa, synthetic construct
DIVMTQSPSSLAMSVGQKVTMSCKSSQSLLNSSNQKNHLAWYQQKPGQSPKLLVYFASTRGSGVPDRFIGSGSGTDFTLTISSVQAEDLADYFCQQHYSTPLTFGAGTKLELK

SEQ ID NO: 135 - protein, 114 aa, synthetic construct; identical to SEQ ID NO: 131

SEQ ID NO: 136 - protein, 113 aa, synthetic construct
DIVMTQSPSSLAMSVGQKVTMSCKSSQSLLNSSNQKNYLAWYQQKPGQSPKLLVYFASTRDSGVPDRFIGSGSGTDFTLTISSVQAEDLADYFCQQHYSTPLTFGAGTKLELK

SEQ ID NO: 137 - protein, 114 aa, synthetic construct; identical to SEQ ID NO: 131

SEQ ID NO: 138 - protein, 113 aa, synthetic construct
DIVMTQSPSSLAMSVGQKVTMSCKSSQSLLNSSNQKNYLAWYQQKPGQSPKLLVYFASTRESGVPDRFIGSGSGTDFTLTISSVQAEDLADYFCQQHYSTPLTFGAGTKLELK

SEQ ID NO: 139 - protein, 119 aa, synthetic construct
EVMLVESGGGLVKPGGSLKLSCAASRFTFSNYAMSWVRQTPEKRLEWVATITSGGSYTYYPDSVKGRFTISRDNAKNTLYLQMSSLRSEDTAMYYCARKDYGNYWFAYWGQGTLVTVSA

SEQ ID NO: 140 - protein, 112 aa, synthetic construct
DVVMTQTPLSLPVSLGDQASISCRSSQSLVHSDGNTYLHWYLQKPGQSPKLLIYKVSNRFSGVPDRFSGSGSGTDFTLKISRVEAEDLGVYFCSQSIHVPWTFGGGTKLEIK

SEQ ID NO: 141 - protein, 119 aa, synthetic construct
EVLLVESGGGLVKPGGSLKLSCAASGFTFSGYAMSWVRQTPEKRLEWVATITSGGSYTYYPDSVKGRFTISRDNAKNTLYLQMSSLRSEDTAMYYCARKDYGNYWFAYWGQGTLVTVSA

SEQ ID NO: 142 - protein, 106 aa, synthetic construct
QIVLTQSPAIMSASPGEKVTITCSASSSVSYMHWFQQKPGTSPKLWIYSTSNLASGVPARFSGSGSGTSYSLTISRMEAEDAATYYCQQRSSYPLTVGAGTKLELK

SEQ ID NO: 143 - protein, 119 aa, synthetic construct; identical to SEQ ID NO: 141

SEQ ID NO: 144 - protein, 112 aa, synthetic construct
DVVMTQTPLSLPVSLGDQASISCRSSQSLVHSDGNTYLHWYLQKPGQSPKLLIYKVSNRFSGVPDRFSGSGSGTDFTLKISRVEAEDLGVYFCSQTTQVPWTFGGGTKLEIK

SEQ ID NO: 145 - protein, 119 aa, synthetic construct
DVQLQESGPDLVKPSQSLSLNCTVTGYSITSGYSWHWIRQFPGNKLEWMGYIHYSGSTNYNPPLKSRIFIARDTSKNQFFLQLTSVTTEDTATYYCARGVVSNYAMGNWGQGTSVTVSS

SEQ ID NO: 146 - protein, 107 aa, synthetic construct
ETTVTQSPASLSMAIGEKVTIRCITNTDIDDDMNWYQQKPGEPPKLLISEGNTLRPGVPSRFSSSGYGTDFVFTIENMLSEDVADYYCLQSDDLPLTFGSGTKLEIK

SEQ ID NO: 147 - protein, 121 aa, synthetic construct
QVQLQQSGAELAKPGASVKMSCKASAYTFTTYWMHWVKQRPGQGLEWIGYINPNTAYTEYNQNFKDKATLTADKSSSTAYMQLGSLTSEDSAVYYCARGAYYRTYYAMDYWGQGTSVTVSS

SEQ ID NO: 148 - protein, 111 aa, synthetic construct
DIVLTQSPASLAVSLGQRATISCKASQSVDYDGDSYMNWYQQKPGQPPKLLIYAASNLESGIPARFSGSGSGTDFTLNIHPVEEEDAATYYCLQSNEDPYTFGGGTRLEIN

SEQ ID NO: 149 - protein, 120 aa, synthetic construct
QIQLVQSGPELKKPGETVKISCKASGYTFINYGMNWVKQTPGKGLKWMGWINTYTGEPTYADDFKGRFAFSLETSASTAYLQINNLKNEDMATYFCSREEFYSRGAMDYWGQGTSVTVSS

SEQ ID NO: 150 - protein, 112 aa, synthetic construct
DVLMTQTPLSLPVSLGDQASISCRSSQFIVHSNGNTYLEWYLQKPGQSPKLLIYKISNRFSGVPDRFSGSGSGTDFTLKISRVEAEDLGVYYCFQGSHVPFTFGSGTKLEIK

SEQ ID NO: 151 - protein, 115 aa, synthetic construct
QIQLQQSGPELVKPGASVKISCKASGYSFTDYYINWVKQKPGQGLEWIGWIYPGSGNTKYNEKFKGKATLTVDTSSSTAYMQLNSLTSEDTAVYFCARSSRCDFWGQGTTLTVSS

SEQ ID NO: 152 - protein, 107 aa, synthetic construct
DIQMTQSASSFSVSLGDSVTITCKASEDIYNRLAWYQQKPGNTPRLLISGATSLETGVPSRFSGSGSGKDYTLSITSLQTEDVATYYCQQYWSSPLTFGSGTKLELK

SEQ ID NO: 153 - DNA, 63 bp, synthetic construct
  source 1..63: mol_type = other DNA
atggccctccctgtcaccgccctgctgcttccgctggctcttctgctccacgccgctcggccc

SEQ ID NO: 154 - protein, 21 aa, synthetic construct
MALPVTALLLPLALLLHAARP

SEQ ID NO: 155 - DNA, 135 bp, synthetic construct
  source 1..135: mol_type = other DNA
accacgacgccagcgccgcgaccaccaacaccggcgcccaccatcgcgtcgcagcccctgtccctgcgcccagaggcgtgccggccagcggcggggggcgcagtgcacacgagggggctggacttcgcctgtgat

SEQ ID NO: 156 - protein, 45 aa, synthetic construct
TTTPAPRPPTPAPTIASQPLSLRPEACRPAAGGAVHTRGLDFACD

SEQ ID NO: 157 - DNA, 72 bp, synthetic construct
  source 1..72: mol_type = other DNA
atctacatctgggcgcccttggccgggacttgtggggtccttctcctgtcactggttatcaccctttactgc

SEQ ID NO: 158 - protein, 24 aa, synthetic construct
IYIWAPLAGTCGVLLLSLVITLYC

SEQ ID NO: 159 - DNA, 126 bp, synthetic construct
  source 1..126: mol_type = other DNA
aaacggggcagaaagaaactcctgtatatattcaaacaaccatttatgagaccagtacaaactactcaagaggaagatggctgtagctgccgatttccagaagaagaagaaggaggatgtgaactg

SEQ ID NO: 160 - protein, 42 aa, synthetic construct
KRGRKKLLYIFKQPFMRPVQTTQEEDGCSCRFPEEEEGGCEL

SEQ ID NO: 161 - DNA, 120 bp, synthetic construct
  source 1..120: mol_type = other DNA
tctaagcggtccagactgctccacagtgattacatgaacatgaccccacgcaggcctgggccaacacgaaaacactatcagccttacgcacctccccgcgactttgctgcctaccgctct

SEQ ID NO: 162 - protein, 40 aa, synthetic construct
SKRSRLLHSDYMNMTPRRPGPTRKHYQPYAPPRDFAAYRS

SEQ ID NO: 163 - DNA, 336 bp, synthetic construct
  source 1..336: mol_type = other DNA
agagtgaagttcagcaggagcgcagacgcccccgcgtacaagcagggccagaaccagctctataacgagctcaatctaggacgaagagaggagtacgatgttttggacaagagacgtggccgggaccctgagatggggggaaagccgagaaggaagaaccctcaggaaggcctgtacaatgaactgcagaaagataagatggcggaggcctacagtgagattgggatgaaaggcgagcgccggaggggcaaggggcacgatggcctttaccagggtctcagtacagccaccaaggacacctacgacgcccttcacatgcaggccctgccccctcgc

SEQ ID NO: 164 - protein, 112 aa, synthetic construct
RVKFSRSADAPAYKQGQNQLYNELNLGRREEYDVLDKRRGRDPEMGGKPRRKNPQEGLYNELQKDKMAEAYSEIGMKGERRRGKGHDGLYQGLSTATKDTYDALHMQALPPR

SEQ ID NO: 165 - DNA, 60 bp, synthetic construct
  source 1..60: mol_type = other DNA
ggcggaggcgggtcaggaggtggcggcagcggaggaggagggtccggcggaggtgggtcc

SEQ ID NO: 166 - protein, 20 aa, synthetic construct
GGGGSGGGGSGGGGSGGGGS

SEQ ID NO: 167 - protein, 247 aa, synthetic construct
QVQLVQSGAEVKKPGASVKVSCKASGFNIKDYYMHWVRQAPGQRLEWIGWIDPENGNTIYDPKFQGRATITADTSASTAYMELSSLRSEDTAVYYCARGWFAYWGQGTLVTVSSGGGGSGGGGSGGGGSGGGGSDIVMTQSPDSLAVSLGERATINCKSSQSLLNSSNQKNHLAWYQQKPGQPPKLLIYFASTRASGVPDRFSGSGSGTDFTLTISSLQAEDVAVYYCQQHYSTPLTFGGGTKLELK

SEQ ID NO: 168 - DNA, 741 bp, synthetic construct
  source 1..741: mol_type = other DNA
caagtgcagctggtgcagtccggcgctgaagtgaagaagcccggcgcctccgtgaaagtgtcctgcaaggcctctggcttcaacatcaaggactactatatgcactgggtgcggcaggctcctggccagcggctggagtggatcggctggatcgaccctgagaacggcaacaccatctacgaccccaagttccagggcagagccaccatcaccgccgacaccagcgccagcactgcttatatggaactgagctctctgagaagcgaggataccgctgtctactactgtgccagaggctggttcgcctactggggccaaggcaccctcgtcacagtgtctagcggagggggcggatctgggggcggcggctccggaggaggcggttctggcggtggcggctcggacatcgtgatgacacagtctcctgatagcctggctgtgtccctgggcgagcgggcaaccatcaactgcaagtccagccagagcctgctgaacagcagcaatcagaagaaccacctggcctggtaccagcagaaaccaggccagcctcctaagctgctgatttactttgcctctaccagagccagcggcgtgcccgatagattcagcggctccggatccggcaccgacttcaccctgacaatctctagcctgcaggccgaggacgtggccgtgtactactgccagcagcactactccacccctctgaccttcggcggcggaacaaagctggaactgaag

SEQ ID NO: 169 - protein, 247 aa, synthetic construct
QVQLVQSGAEVKKPGASVKVSCKASGFNIKDYYMHWVRQAPGQRLEWIGWIDPENGNTIYDPKFQGRATITADTSASTAYMELSSLRSEDTAVYYCARGWFAYWGQGTLVTVSSGGGGSGGGGSGGGGSGGGGSDIVMTQSPDSLAVSLGERATINCKSSQSLLNSSNQKNHLAWYQQKPGQPPKLLVYFASTRASGVPDRFSGSGSGTDFTLTISSLQAEDVAVYFCQQHYSTPLTFGGGTKLELK

SEQ ID NO: 170 - DNA, 741 bp, synthetic construct
  source 1..741: mol_type = other DNA
caagtgcagctggtgcagtctggggccgaggtgaagaagcccggcgctagcgtgaaagtgtcctgcaaggctagcggcttcaacatcaaggactactacatgcactgggtgcggcaggcccctggacagagactggaatggatcggctggatcgaccccgagaacggcaacaccatctacgaccctaagttccagggcagagccacaatcaccgccgatacaagcgcctctactgcctacatggaactgagctctctgcggtctgaagataccgctgtctactactgcgccagaggctggttcgcctactggggccagggcacactggtgacagtgtcctcgggcggtggaggctccggcggcggcggctctggcggcggtggcagcggaggaggcggatccgacatcgtgatgacccagtcccccgacagcctggctgtgtctctgggcgagcgggccaccatcaactgcaagtcctctcagtccctgctgaacagcagcaatcagaagaaccacctggcctggtaccagcaaaaacctggccagcctccaaagctgctggtctattttgcttctaccagagcctccggcgtgcctgatagattctccggcagcggctccggcaccgacttcaccctcaccatcagcagcctgcaggctgaggacgtggccgtgtacttctgtcagcagcactacagcacccctctgaccttcggcggaggcaccaagctggagctgaag

SEQ ID NO: 171 - protein, 247 aa, synthetic construct
QVQLVQSGAEVKKPGASVKVSCKASGFNIKDYYMHWVKQAPGQRLEWIGWIDPENGNTIYDPKFQGRATITADTSANTAYMELSSLRSEDTAVYYCARGWFAYWGQGTLVTVSSGGGGSGGGGSGGGGSGGGGSDIVMTQSPDSLAVSLGERATINCKSSQSLLNSSNQKNHLAWYQQKPGQPPKLLIYFASTRASGVPDRFSGSGSGTDFTLTISSLQAEDVAVYYCQQHYSTPLTFGGGTKLELK

SEQ ID NO: 172 - DNA, 741 bp, synthetic construct
  source 1..741: mol_type = other DNA
caagtgcagctcgtccagtctggcgccgaagtgaagaagcccggcgcttccgtgaaagtgtcctgcaaggcctctggcttcaacatcaaggactactacatgcactgggtcaagcaggcccctggccagcggctggaatggattggctggatcgaccctgagaacggcaacaccatctacgaccccaagttccagggcagagccactatcaccgccgatacaagcgccaatacagcttatatggaactgtcctccctgagaagcgaggatacagccgtgtactactgcgccagaggctggttcgcctactggggccaaggcaccctggtgaccgtgtcttctggcggcggcggctctggcggcggaggatctggcggaggcggcagtggcggaggcggaagcgacatcgtgatgacccagtccccagattccctggccgtgtctctgggcgagcgggctaccatcaactgcaagtccagccagagcctgctgaacagcagcaaccagaagaaccacctggcctggtaccagcagaaacccggccagcctcctaagctgctgatctactttgcttccaccagagctagcggcgtgcctgaccggttcagcggctccggttctggaacagacttcaccctgaccatcagctccctgcaggccgaggacgtggccgtgtactactgtcagcagcactacagcacccctctgaccttcggcggcggcaccaagctggagctgaag

SEQ ID NO: 173 - protein, 247 aa, synthetic construct
QVQLVQSGAEVKKPGASVKVSCKASGFNIKDYYMHWVRQAPGQRLEWIGWIDPENGNTIYDPKFQGRATITADTSASTAYMELSSLRSEDTAVYYCARGWFAYWGQGTLVTVSSGGGGSGGGGSGGGGSGGGGSDIVMTQSPDSLAVSLGERATINCKSSQSLLNSSNQKNHLAWYQQKPGQPPKLLIYFASTRGSGVPDRFSGSGSGTDFTLTISSLQAEDVAVYYCQQHYSTPLTFGGGTKLELK

SEQ ID NO: 174 - DNA, 741 bp, synthetic construct
  source 1..741: mol_type = other DNA
caagtgcagctggtgcagtccggcgctgaagtgaagaagcccggcgcctccgtgaaagtgtcctgcaaggcctctggcttcaacatcaaggactactatatgcactgggtgcggcaggctcctggccagcggctggagtggatcggctggatcgaccctgagaacggcaacaccatctacgaccccaagttccagggcagagccaccatcaccgccgacaccagcgccagcactgcttatatggaactgagctctctgagaagcgaggataccgctgtctactactgtgccagaggctggttcgcctactggggccaaggcaccctcgtcacagtgtctagcggagggggcggatctgggggcggcggctccggaggaggcggttctggcggtggcggctcggacatcgtgatgacacagtctcctgatagcctggctgtgtccctgggcgagcgggcaaccatcaactgcaagtccagccagagcctgctgaacagcagcaatcagaagaaccacctggcctggtaccagcagaaaccaggccagcctcctaagctgctgatttactttgcctctaccagaggcagcggcgtgcccgatagattcagcggctccggatccggcaccgacttcaccctgacaatctctagcctgcaggccgaggacgtggccgtgtactactgccagcagcactactccacccctctgaccttcggcggcggaacaaagctggaactgaag

SEQ ID NO: 175 - protein, 247 aa, synthetic construct
QVQLVQSGAEVKKPGASVKVSCKASGFNIKDYYMHWVRQAPGQRLEWIGWIDPENGNTIYDPKFQGRATITADTSASTAYMELSSLRSEDTAVYYCARGWFAYWGQGTLVTVSSGGGGSGGGGSGGGGSGGGGSDIVMTQSPDSLAVSLGERATINCKSSQSLLNSSNQKNHLAWYQQKPGQPPKLLVYFASTRGSGVPDRFSGSGSGTDFTLTISSLQAEDVAVYFCQQHYSTPLTFGGGTKLELK

SEQ ID NO: 176 - DNA, 741 bp, synthetic construct
  source 1..741: mol_type = other DNA
caagtgcagctggtgcagtctggggccgaggtgaagaagcccggcgctagcgtgaaagtgtcctgcaaggctagcggcttcaacatcaaggactactacatgcactgggtgcggcaggcccctggacagagactggaatggatcggctggatcgaccccgagaacggcaacaccatctacgaccctaagttccagggcagagccacaatcaccgccgatacaagcgcctctactgcctacatggaactgagctctctgcggtctgaagataccgctgtctactactgcgccagaggctggttcgcctactggggccagggcacactggtgacagtgtcctcgggcggtggaggctccggcggcggcggctctggcggcggtggcagcggaggaggcggatccgacatcgtgatgacccagtcccccgacagcctggctgtgtctctgggcgagcgggccaccatcaactgcaagtcctctcagtccctgctgaacagcagcaatcagaagaaccacctggcctggtaccagcaaaaacctggccagcctccaaagctgctggtctattttgcttctaccagaggctccggcgtgcctgatagattctccggcagcggctccggcaccgacttcaccctcaccatcagcagcctgcaggctgaggacgtggccgtgtacttctgtcagcagcactacagcacccctctgaccttcggcggaggcaccaagctggagctgaag

SEQ ID NO: 177 - protein, 247 aa, synthetic construct
QVQLVQSGAEVKKPGASVKVSCKASGFNIKDYYMHWVKQAPGQRLEWIGWIDPENGNTIYDPKFQGRATITADTSANTAYMELSSLRSEDTAVYYCARGWFAYWGQGTLVTVSSGGGGSGGGGSGGGGSGGGGSDIVMTQSPDSLAVSLGERATINCKSSQSLLNSSNQKNHLAWYQQKPGQPPKLLIYFASTRGSGVPDRFSGSGSGTDFTLTISSLQAEDVAVYYCQQHYSTPLTFGGGTKLELK

SEQ ID NO: 178 - DNA, 741 bp, synthetic construct
  source 1..741: mol_type = other DNA
caagtgcagctcgtccagtctggcgccgaagtgaagaagcccggcgcttccgtgaaagtgtcctgcaaggcctctggcttcaacatcaaggactactacatgcactgggtcaagcaggcccctggccagcggctggaatggattggctggatcgaccctgagaacggcaacaccatctacgaccccaagttccagggcagagccactatcaccgccgatacaagcgccaatacagcttatatggaactgtcctccctgagaagcgaggatacagccgtgtactactgcgccagaggctggttcgcctactggggccaaggcaccctggtgaccgtgtcttctggcggcggcggctctggcggcggaggatctggcggaggcggcagtggcggaggcggaagcgacatcgtgatgacccagtccccagattccctggccgtgtctctgggcgagcgggctaccatcaactgcaagtccagccagagcctgctgaacagcagcaaccagaagaaccacctggcctggtaccagcagaaacccggccagcctcctaagctgctgatctactttgcttccaccagaggtagcggcgtgcctgaccggttcagcggctccggttctggaacagacttcaccctgaccatcagctccctgcaggccgaggacgtggccgtgtactactgtcagcagcactacagcacccctctgaccttcggcggcggcaccaagctggagctgaag

SEQ ID NO: 179 - protein, 251 aa, synthetic construct
EVQLLESGGGLVQPGGSLKLSCAASGFTFSGYAMSWVRQTPGKGLEWVATITSGGSYTYYPDSVKGRFTISRDNSKNTLYLQMNSLRAEDTAMYYCARKDYGNYWFAYWGQGTLVTVSSGGGGSGGGGSGGGGSGGGGSDVVMTQSPLSLPVTLGDPASISCRSSQSLVHSDGNTYLHWYLQRPGQSPRLLIYKVSNRFSGVPDRFSGSGSGTDFTLKISRVEAEDVGVYFCSQTTQVPWTFGGGTKLEIK

SEQ ID NO: 180 - DNA, 753 bp, synthetic construct
  source 1..753: mol_type = other DNA
gaggtgcagctgctggaaagcggcggaggactggtgcaacctggaggatctctgaagctgagctgcgccgcttctggctttacattcagcggctacgccatgagctgggtcagacagacccctggcaagggcctcgagtgggtggccacaatcaccagcggcggcagctacacctactaccccgacagcgtgaaaggcagattcaccatcagccgggacaattctaagaacaccctgtacctgcagatgaactccctgcgggccgaagataccgccatgtactattgtgctagaaaggactacggcaactactggttcgcctactggggccagggcaccctggtgacagtgtccagcggcggcggcggctctggcggcggcggaagcggcggcgggggttccggcggaggaggctccgatgtggtgatgacccaaagccctctgagcctgcctgtgaccctgggcgaccccgccagcatctcttgtagaagcagccagtccctcgtgcacagcgacggcaacacctacctgcactggtacctgcagcggcctggccagtctccaagactgctgatctataaggtgtccaaccggttcagcggagttcctgatagatttagcggcagcggctctggaacagacttcacactgaaaatctctagagtggaggccgaggacgtgggcgtctacttctgcagccagaccacacaggtgccctggaccttcggcggaggcaccaagctggaaatcaag

SEQ ID NO: 181 - protein, 251 aa, synthetic construct
EVQLLESGGGLVQPGGSLKLSCAASGFTFSGYAMSWVRQTPGKGLEWVATITSGGSYTYYPDSVKGRFTISRDNSKNTLYLQMNSLRAEDTAMYYCARKDYGNYWFAYWGQGTLVTVSSGGGGSGGGGSGGGGSGGGGSDVVMTQSPLSLPVTLGQQASISCRSSQSLVHSDGNTYLHWYLQKPGQSPKLLIYKVSNRFSGVPDRFSGSGSGTDFTLKISRVEAEDVGVYFCSQTTQVPWTFGGGTKLEIK

SEQ ID NO: 182 - DNA, 753 bp, synthetic construct
  source 1..753: mol_type = other DNA
gaggtgcagctgctggaaagcggcggaggactggtgcaacctggaggatctctgaagctgagctgcgccgcttctggctttacattcagcggctacgccatgagctgggtcagacagacccctggcaagggcctcgagtgggtggccacaatcaccagcggcggcagctacacctactaccccgacagcgtgaaaggcagattcaccatcagccgggacaattctaagaacaccctgtacctgcagatgaactccctgcgggccgaagataccgccatgtactattgtgctagaaaggactacggcaactactggttcgcctactggggccagggcaccctggtgacagtgtccagcggcggcggcggctctggcggcggcggaagcggcggcgggggttccggcggaggaggctccgacgtcgtgatgacacagagccccctgagcctgcctgtgaccctgggccagcaggccagcatcagctgtagaagcagccagtccctggtgcactccgacggcaacacctacctgcactggtacctgcagaaacctggccagtctccaaagctgctgatctacaaggtgtccaaccggtttagcggcgttcctgatagattcagcggatctggcagcggcacagatttcaccctgaagatctctagagtggaagccgaggacgtgggcgtgtatttctgcagccagaccacccaagtgccctggaccttcggcggaggcacaaagctcgagatcaag

SEQ ID NO: 183 - protein, 251 aa, synthetic construct
EVQLLESGGGLVQPGGSLKLSCAASGFTFSGYAMSWVRQTPGKGLEWVATITSGGSYTYYPDSVKGRFTISRDNSKNTLYLQMNSLRAEDTAMYYCARKDYGNYWFAYWGQGTLVTVSSGGGGSGGGGSGGGGSGGGGSDVVMTQSPLSLPVTLGDQASISCRSSQSLVHSDGNTYLHWYLQKPGQSPKLLIYKVSNRFSGVPDRFSGSGSGTDFTLKISRVEAEDVGVYFCSQTTQVPWTFGGGTKLEIK

SEQ ID NO: 184 - DNA, 753 bp, synthetic construct
  source 1..753: mol_type = other DNA
gaggtgcagctgctggaaagcggcggaggactggtgcaacctggaggatctctgaagctgagctgcgccgcttctggctttacattcagcggctacgccatgagctgggtcagacagacccctggcaagggcctcgagtgggtggccacaatcaccagcggcggcagctacacctactaccccgacagcgtgaaaggcagattcaccatcagccgggacaattctaagaacaccctgtacctgcagatgaactccctgcgggccgaagataccgccatgtactattgtgctagaaaggactacggcaactactggttcgcctactggggccagggcaccctggtgacagtgtccagcggcggcggcggctctggcggcggcggaagcggcggcgggggttccggcggaggaggctccgatgtggtgatgacccagtccccactgagcctgcctgtgaccctgggcgaccaggccagcatcagctgtagaagcagccaatctctggtgcacagcgacggcaacacatacctgcactggtatctgcagaaacctggccagagccccaagctgctgatctacaaggtgtccaaccggtttagcggagtgcctgatagattcagcggctctggctccggcaccgacttcaccctcaagatctctagagtcgaggccgaggacgtgggcgtgtacttctgcagccagaccacacaggtgccctggaccttcggcggcggaacaaagctggaaatcaag

SEQ ID NO: 185 - protein, 251 aa, synthetic construct
EVQLLESGGGLVQPGGSLKLSCAASGFTFSGYAMSWVRQTPEKGLEWVATITSGGSYTYYPDSVKGRFTISRDNAKNTLYLQMNSLRAEDTAMYYCARKDYGNYWFAYWGQGTLVTVSSGGGGSGGGGSGGGGSGGGGSDVVMTQSPLSLPVTLGDPASISCRSSQSLVHSDGNTYLHWYLQRPGQSPRLLIYKVSNRFSGVPDRFSGSGSGTDFTLKISRVEAEDVGVYFCSQTTQVPWTFGGGTKLEIK

SEQ ID NO: 186 - DNA, 753 bp, synthetic construct
  source 1..753: mol_type = other DNA
gaggtgcagctgctggaaagcggcggcggactcgtgcaacctggcggatctctgaagctgtcttgtgctgcttctggatttaccttcagcggctacgccatgagctgggtgcggcagacacctgagaagggcctggaatgggtcgccacaatcaccagcggcggctcctacacctactaccccgatagcgtgaaaggcagattcacaatcagccgggacaacgccaagaacaccctgtacctgcagatgaacagcctgagagccgaggacaccgccatgtactactgcgccagaaaggactacggcaattactggttcgcctattggggccagggcaccctggtgaccgtgtccagcggcggcggcggctctggcggcggcggaagcggcggcgggggttccggcggaggaggctccgatgtggtgatgacccaaagccctctgagcctgcctgtgaccctgggcgaccccgccagcatctcttgtagaagcagccagtccctcgtgcacagcgacggcaacacctacctgcactggtacctgcagcggcctggccagtctccaagactgctgatctataaggtgtccaaccggttcagcggagttcctgatagatttagcggcagcggctctggaacagacttcacactgaaaatctctagagtggaggccgaggacgtgggcgtctacttctgcagccagaccacacaggtgccctggaccttcggcggaggcaccaagctggaaatcaag

SEQ ID NO: 187 - protein, 251 aa, synthetic construct
EVQLLESGGGLVQPGGSLKLSCAASGFTFSGYAMSWVRQTPEKGLEWVATITSGGSYTYYPDSVKGRFTISRDNAKNTLYLQMNSLRAEDTAMYYCARKDYGNYWFAYWGQGTLVTVSSGGGGSGGGGSGGGGSGGGGSDVVMTQSPLSLPVTLGQQASISCRSSQSLVHSDGNTYLHWYLQKPGQSPKLLIYKVSNRFSGVPDRFSGSGSGTDFTLKISRVEAEDVGVYFCSQTTQVPWTFGGGTKLEIK

SEQ ID NO: 188 - DNA, 753 bp, synthetic construct
  source 1..753: mol_type = other DNA
gaggtgcagctgctggaaagcggcggcggactcgtgcaacctggcggatctctgaagctgtcttgtgctgcttctggatttaccttcagcggctacgccatgagctgggtgcggcagacacctgagaagggcctggaatgggtcgccacaatcaccagcggcggctcctacacctactaccccgatagcgtgaaaggcagattcacaatcagccgggacaacgccaagaacaccctgtacctgcagatgaacagcctgagagccgaggacaccgccatgtactactgcgccagaaaggactacggcaattactggttcgcctattggggccagggcaccctggtgaccgtgtccagcggcggcggcggctctggcggcggcggaagcggcggcgggggttccggcggaggaggctccgacgtcgtgatgacacagagccccctgagcctgcctgtgaccctgggccagcaggccagcatcagctgtagaagcagccagtccctggtgcactccgacggcaacacctacctgcactggtacctgcagaaacctggccagtctccaaagctgctgatctacaaggtgtccaaccggtttagcggcgttcctgatagattcagcggatctggcagcggcacagatttcaccctgaagatctctagagtggaagccgaggacgtgggcgtgtatttctgcagccagaccacccaagtgccctggaccttcggcggaggcacaaagctcgagatcaag

SEQ ID NO: 189 - protein, 251 aa, synthetic construct
EVQLLESGGGLVQPGGSLKLSCAASGFTFSGYAMSWVRQTPEKGLEWVATITSGGSYTYYPDSVKGRFTISRDNAKNTLYLQMNSLRAEDTAMYYCARKDYGNYWFAYWGQGTLVTVSSGGGGSGGGGSGGGGSGGGGSDVVMTQSPLSLPVTLGDQASISCRSSQSLVHSDGNTYLHWYLQKPGQSPKLLIYKVSNRFSGVPDRFSGSGSGTDFTLKISRVEAEDVGVYFCSQTTQVPWTFGGGTKLEIK

SEQ ID NO: 190 - DNA, 753 bp, synthetic construct
  source 1..753: mol_type = other DNA
gaggtgcaactgctggaatccggcggcggactggtgcagcccggcggctctctgaagctgagctgtgctgcttctggctttaccttcagcggctacgccatgagctgggtcagacagacacctgagaagggcctggaatgggtggccacaatcaccagcggaggatcttatacatactaccctgatagcgtgaaaggcagattcaccatcagccgggacaacgccaagaacaccctgtacctgcagatgaacagcctgcgggccgaggacaccgccatgtactactgcgccagaaaggactacggcaattactggttcgcctactggggccagggcaccctcgtgaccgtgtccagcggcggcggcggctctggcggcggcggaagcggcggcgggggttccggcggaggaggctccgatgtggttatgacccagtctccactgagcctgcctgtgacactgggagatcaggccagcatcagctgtagaagcagccagtccctggtgcacagcgacggcaacacctacctgcactggtatctgcagaaacctggccagagccccaagctgctgatctacaaggtgtccaaccggtttagcggcgtgcccgacagattctccggcagcggatctggcaccgacttcaccctgaagatctctagagtggaagccgaggacgtgggcgtctacttctgcagccagaccacccaagtgccttggacattcggcggcggaacaaagctcgagatcaag

SEQ ID NO: 191 - protein, 18 aa, synthetic construct
EGRGSLLTCGDVEENPGP

SEQ ID NO: 192 - DNA, 54 bp, synthetic construct
  source 1..54: mol_type = other DNA
gagggcagaggaagtcttctaacatgcggtgacgtggaggagaatcccggccct

SEQ ID NO: 193 - protein, 166 aa, synthetic construct
MGRGLLRGLWPLHIVLWTRIASTIPPHVQKSVNNDMIVTDNNGAVKFPQLCKFCDVRFSTCDNQKSCMSNCSITSICEKPQEVCVAVWRKNDENITLETVCHDPKLPYHDFILEDAASPKCIMKEKKKPGETFFMCSCSSDECNDNIIFSEEYNTSNPDLLLVIFQ

SEQ ID NO: 194 - DNA, 597 bp, synthetic construct
  source 1..597: mol_type = other DNA
atgggtcgggggctgctcaggggcctgtggccgctgcacatcgtcctgtggacgcgtatcgccagcacgatcccaccgcacgttcagaagtcggatgtggaaatggaggcccagaaagatgaaatcatctgccccagctgtaataggactgcccatccactgagacatattaataacgacatgatagtcactgacaacaacggtgcagtcaagtttccacaactgtgtaaattttgtgatgtgagattttccacctgtgacaaccagaaatcctgcatgagcaactgcagcatcacctccatctgtgagaagccacaggaagtctgtgtggctgtatggagaaagaatgacgagaacataacactagagacagtttgccatgaccccaagctcccctaccatgactttattctggaagatgctgcttctccaaagtgcattatgaaggaaaaaaaaaagcctggtgagactttcttcatgtgttcctgtagctctgatgagtgcaatgacaacatcatcttctcagaagaatataacaccagcaatcctgacttgttgctagtcatatttcaagtgacaggcatcagcctcctgcca

SEQ ID NO: 195 - protein, 25 aa, synthetic construct
PILLTISILSFFSVALLVILACVLW

SEQ ID NO: 196 - DNA, 75 bp, synthetic construct
  source 1..75: mol_type = other DNA
ccaattctgctgaccatttcaatcctttcctttttctccgtggctctcctggtgattctggcatgcgtgctgtgg

SEQ ID NO: 197 - protein, 195 aa, synthetic construct
KKRIKPIVWPSLPDHKKTLEHLCKKPRKNLNVSFNPESFLDCQIHRVDDIQARDEVEGFLQDTFPQQLEESEKQRLGGDVQSPNCPSEDVVITPESFGRDSSLTCLAGNVSACDAPILSSSRSLDCRESGKNGPHVYQDLLLSLGTTNSTLPPPFSLQSGILTLNPVAQGQPILTSLGSNQEEAYVTMSSFYQNQ

SEQ ID NO: 198 - DNA, 585 bp, synthetic construct
  source 1..585: mol_type = other DNA
aagaagcgcatcaagcccatcgtttggccctctcttcccgatcacaagaagaccctggagcacctgtgcaagaagccgcgcaagaacctcaacgtgtccttcaacccagagtccttcctggactgtcaaatccaccgcgtcgatgacatccaggcccgtgatgaagtcgagggctttctgcaggacacgttcccgcaacagctagaagagtcggagaagcagcgcctgggtggtgatgtgcagagccctaactgcccatcggaagatgtggtcatcaccccggagagcttcggccgggattcctctttgacttgcctggccgggaacgtgtccgcgtgcgacgcgcccatcctatcctcctccagatctctggactgtagggagtctggcaaaaacggacctcacgtatatcaggacctgttgctgagcctgggaaccaccaactcgacccttcctccgcccttctccttacagtccggcatcctgaccctcaaccctgttgcccagggccagccgatcctcacttcactgggctccaaccaggaggaggcctacgtgaccatgtctagcttctaccagaaccag